European Patent Specification EP 4 363 850 B1, published August 20, 2025. Title: PHOTO-ELECTROCHEMICAL PARTICLE ASSAY. Applicant: Universiteit Antwerpen. The sequence listing filed with the application follows.

SEQUENCE LISTING (14 sequences)

SEQ ID NO: 1 - DNA, 12 bp, Artificial Sequence
  Detection of miR-145
ggaaaactggac

SEQ ID NO: 2 - DNA, 11 bp, Artificial Sequence
  Capture miR-145
agggattcctg

SEQ ID NO: 3 - RNA, 23 nt, Artificial Sequence
  Target miR-145
guccaguuuucccaggaaucccu

SEQ ID NO: 4 - DNA, 11 bp, Artificial Sequence
  Detection of miR-141
agacagtgtta

SEQ ID NO: 5 - DNA, 11 bp, Artificial Sequence
  Capture miR-141
ccatctttacc

SEQ ID NO: 6 - RNA, 22 nt, Artificial Sequence
  Target miR-141
uaacacugucugguaaagaugg

SEQ ID NO: 7 - DNA, 12 bp, Artificial Sequence
  Detection miR-375
cgaacgaacaaa

SEQ ID NO: 8 - DNA, 10 bp, Artificial Sequence
  Capture miR-375
tcacgcgagc

SEQ ID NO: 9 - RNA, 21 nt, Artificial Sequence
  Target miR-375
uuuguucguucgcucgcguga

SEQ ID NO: 10 - DNA, 18 bp, Artificial Sequence
  Detection sequence complementary to miR-21
tcaacatcagtctgataa

SEQ ID NO: 11 - DNA, 22 bp, Artificial Sequence
  Capture sequence complementary to miR-21
tagcttatcagactgatgttga

SEQ ID NO: 12 - DNA, 17 bp, Artificial Sequence
  Detection  sequence complementary to KRAS G12C
cgtcaaggcactcttgc

SEQ ID NO: 13 - DNA, 17 bp, Artificial Sequence
  Capture sequence complementary to KRAS G12C
ctacgccacaagctcca

SEQ ID NO: 14 - DNA, 34 bp, Artificial Sequence
  Target sequence KRASG12C
tggagcttgtggcgtaggcaagagtgccttgacg